European Patent Application EP 4 410 309 A1, published August 7, 2024. Title: Composition containing monoclonal antibody. Applicant: Igalphan corporation. Application EP 22876588.9, filed September 30, 2022. The sequence listing filed with the application follows.

SEQUENCE LISTING (113 sequences)

SEQ ID NO: 1 - protein, 5 aa, Mus musculus
SYGIS

SEQ ID NO: 2 - protein, 16 aa, Mus musculus
EIYPRSGNTYYNEKFK

SEQ ID NO: 3 - protein, 8 aa, Mus musculus
FCARLASS

SEQ ID NO: 4 - protein, 11 aa, Mus musculus
KASQDINSYLS

SEQ ID NO: 5 - protein, 7 aa, Mus musculus
RANRLVD

SEQ ID NO: 6 - protein, 9 aa, Mus musculus
LQYDEFPLT

SEQ ID NO: 7 - protein, 144 aa, Mus musculus
MEWIWIFLFILSGTAGVQSQVQLQQSGAELARPGASVKLSCKASGYTFTSYGISWVKQRTGQGLEWIGEIYPRSGNTYYNEKFKGKATLTADKSSSTAYMELRSLTSEDSAVYFCARLASSYYGSSYDWYFDVWGTGTTVTVSS

SEQ ID NO: 8 - protein, 127 aa, Mus musculus
MRTPAQFLGILLLWFPGIKCDIKMTQSPSSMYASLGERVTITCKASQDINSYLSWFQQKPGKSPKTLIYRANRLVDGVPSRFSGSGSGQDYSLTISSLEYEDMGIYYCLQYDEFPLTFGAGTKLELK

SEQ ID NO: 9 - protein, 488 aa, Mus musculus
MEWIWIFLFILSGTAGVQSQVQLQQSGAELARPGASVKLSCKASGYTFTSYGISWVKQRTGQGLEWIGEIYPRSGNTYYNEKFKGKATLTADKSSSTAYMELRSLTSEDSAVYFCARLASSYYGSSYDWYFDVWGTGTTVTVSSESARNPTIYPLTLPRALSSDPVIIGCLIHDYFPSGTMNVTWGKSGKDITTVNFPPALASGGGYTMSSQLTLPAVECPEGESVKCSVQHDSNAVQELDVKCSGPPPPCPPCPPSCHPSLSLQRPALEDLLLGSDASLTCTLNGLRNPEGAVFTWEPSTGKDAVQKKAVQNSCGCYSVSSVLPGCAERWNSGASFKCTVTHPESDTLTGTIAKITVNTFPPQVHLLPPPSEELALNELVSLTCLVRAFNPKEVLVRWLHGNEELSPESYLVFEPLKEPGEGATTYLVTSVLRVSAELWKQGDQYSCMVGHEALPMNFTQKTIDRLSGKPTNVSVSVIMSEGDGICY

SEQ ID NO: 10 - protein, 234 aa, Mus musculus
MRTPAQFLGILLLWFPGIKCDIKMTQSPSSMYASLGERVTITCKASQDINSYLSWFQQKPGKSPKTLIYRANRLVDGVPSRFSGSGSGQDYSLTISSLEYEDMGIYYCLQYDEFPLTFGAGTKLELKRADAAPTVSIFPPSSEQLTSGGASVVCFLNNFYPKDINVKWKIDGSERQNGVLNSWTDQDSKDSTYSMSSTLTLTKDEYERHNSYTCEATHKTSTSPIVKSFNRNEC

SEQ ID NO: 11 - protein, 5 aa, Mus musculus
TFGMG

SEQ ID NO: 12 - protein, 16 aa, Mus musculus
LAHIWWDDDKYYNPAL

SEQ ID NO: 13 - protein, 8 aa, Mus musculus
YYCARIAG

SEQ ID NO: 14 - protein, 11 aa, Mus musculus
SASSSVSYMHW

SEQ ID NO: 15 - protein, 8 aa, Mus musculus
STSNLASG

SEQ ID NO: 16 - protein, 9 aa, Mus musculus
QRSSYPYTF

SEQ ID NO: 17 - protein, 135 aa, Mus musculus
MGRLTSSFLLLIVPAYVLSQVTLKESGPGILQPSQTLSLTCSFSGFSLSTFGMGVGWIRQPSGKGLEWLAHIWWDDDKYYNPALKSRLTISKDTSKNQVFLKIANVDTADTATYYCARIAGFDYWGQGTTLTVSS

SEQ ID NO: 18 - protein, 128 aa, Mus musculus
MHFQVQIFSFLLISASVIMSRGQIVLTQSPAIMSASPGEKVTITCSASSSVSYMHWFQQKPGTSPKLWIYSTSNLASGVPARFSGSGSGTSYSLTISRMEAEDAATYYCQQRSSYPYTFGGGTKLEIK

SEQ ID NO: 19 - protein, 479 aa, Mus musculus
MGRLTSSFLLLIVPAYVLSQVTLKESGPGILQPSQTLSLTCSFSGFSLSTFGMGVGWIRQPSGKGLEWLAHIWWDDDKYYNPALKSRLTISKDTSKNQVFLKIANVDTADTATYYCARIAGFDYWGQGTTLTVSSESARNPTIYPLTLPRALSSDPVIIGCLIHDYFPSGTMNVTWGKSGKDITTVNFPPALASGGGYTMSSQLTLPAVECPEGESVKCSVQHDSNAVQELDVKCSGPPPPCPPCPPSCHPSLSLQRPALEDLLLGSDASLTCTLNGLRNPEGAVFTWEPSTGKDAVQKKAVQNSCGCYSVSSVLPGCAERWNSGASFKCTVTHPESDTLTGTIAKITVNTFPPQVHLLPPPSEELALNELVSLTCLVRAFNPKEVLVRWLHGNEELSPESYLVFEPLKEPGEGATTYLVTSVLRVSAELWKQGDQYSCMVGHEALPMNFTQKTIDRLSGKPTNVSVSVIMSEGDGICY

SEQ ID NO: 20 - protein, 235 aa, Mus musculus
MHFQVQIFSFLLISASVIMSRGQIVLTQSPAIMSASPGEKVTITCSASSSVSYMHWFQQKPGTSPKLWIYSTSNLASGVPARFSGSGSGTSYSLTISRMEAEDAATYYCQQRSSYPYTFGGGTKLEIKRADAAPTVSIFPPSSEQLTSGGASVVCFLNNFYPKDINVKWKIDGSERQNGVLNSWTDQDSKDSTYSMSSTLTLTKDEYERHNSYTCEATHKTSTSPIVKSFNRNEC

SEQ ID NO: 21 - protein, 5 aa, Mus musculus
SYNIH

SEQ ID NO: 22 - protein, 16 aa, Mus musculus
AIYSGNGATSHNQKFK

SEQ ID NO: 23 - protein, 8 aa, Mus musculus
FCTRVGLR

SEQ ID NO: 24 - protein, 11 aa, Mus musculus
KASQSVGTSVA

SEQ ID NO: 25 - protein, 7 aa, Mus musculus
SASYRYS

SEQ ID NO: 26 - protein, 9 aa, Mus musculus
QQYNNYPYT

SEQ ID NO: 27 - protein, 137 aa, Mus musculus
MGFSRIFLFLLSVTTGVHSQAYLQQSGAELVRPGASVRMSCKASDYTFTSYNIHWVKQTPRQGLEWIGAIYSGNGATSHNQKFKGRATLTVDKSSSTAYMQLSSLTSEDSAVYFCTRVGLRSPFDFWGQGTTLTVSS

SEQ ID NO: 28 - protein, 127 aa, Mus musculus
MESQTQVFVYMLLWLSGVDGDIVMTQSLKFMSTSGGDRVSVTCKASQSVGTSVAWYQQKPGQSPKPLIYSASYRYSGVPDRFTGSGSGTDFSLTISNVQSEDLAEYFCQQYNNYPYTFGGGTKLEIK

SEQ ID NO: 29 - protein, 481 aa, Mus musculus
MGFSRIFLFLLSVTTGVHSQAYLQQSGAELVRPGASVRMSCKASDYTFTSYNIHWVKQTPRQGLEWIGAIYSGNGATSHNQKFKGRATLTVDKSSSTAYMQLSSLTSEDSAVYFCTRVGLRSPFDFWGQGTTLTVSSESARNPTIYPLTLPRALSSDPVIIGCLIHDYFPSGTMNVTWGKSGKDITTVNFPPALASGGGYTMSSQLTLPAVECPEGESVKCSVQHDSNAVQELDVKCSGPPPPCPPCPPSCHPSLSLQRPALEDLLLGSDASLTCTLNGLRNPEGAVFTWEPSTGKDAVQKKAVQNSCGCYSVSSVLPGCAERWNSGASFKCTVTHPESDTLTGTIAKITVNTFPPQVHLLPPPSEELALNELVSLTCLVRAFNPKEVLVRWLHGNEELSPESYLVFEPLKEPGEGATTYLVTSVLRVSAELWKQGDQYSCMVGHEALPMNFTQKTIDRLSGKPTNVSVSVIMSEGDGICY

SEQ ID NO: 30 - protein, 234 aa, Mus musculus
MESQTQVFVYMLLWLSGVDGDIVMTQSLKFMSTSGGDRVSVTCKASQSVGTSVAWYQQKPGQSPKPLIYSASYRYSGVPDRFTGSGSGTDFSLTISNVQSEDLAEYFCQQYNNYPYTFGGGTKLEIKRADAAPTVSIFPPSSEQLTSGGASVVCFLNNFYPKDINVKWKIDGSERQNGVLNSWTDQDSKDSTYSMSSTLTLTKDEYERHNSYTCEATHKTSTSPIVKSFNRNEC

SEQ ID NO: 31 - protein, 5 aa, Mus musculus
DYYIH

SEQ ID NO: 32 - protein, 16 aa, Mus musculus
RIDPENDETTYAPKFQ

SEQ ID NO: 33 - protein, 8 aa, Mus musculus
YCARSTVL

SEQ ID NO: 34 - protein, 11 aa, Mus musculus
RASQSIVHTNG

SEQ ID NO: 35 - protein, 7 aa, Mus musculus
KLLIYKV

SEQ ID NO: 36 - protein, 9 aa, Mus musculus
GVYYCFQGS

SEQ ID NO: 37 - protein, 134 aa, Mus musculus
MKCSWIIFFLMAVVTGVNSEVQLQQSGSELVKSGASVKLSCTVSGFNFTDYYIHWVRQRTEQGLEWIGRIDPENDETTYAPKFQGKATMTADTSSNTAYLQLTSLTSEDTAVYYCARSTVLDYWGHGTTLTVSS

SEQ ID NO: 38 - protein, 131 aa, Mus musculus
MKLPVRLLVLMFWIPGFSSDVLMTQTPLSLPVSLGDQASISCRASQSIVHTNGNTYLEWYLQKPGQSPKLLIYKVSNRFSGVPDRFSGSGSGTDFILKISRVEAEDLGVYYCFQGSHVPPTFGGGTKLEVK

SEQ ID NO: 39 - protein, 478 aa, Mus musculus
MKCSWIIFFLMAVVTGVNSEVQLQQSGSELVKSGASVKLSCTVSGFNFTDYYIHWVRQRTEQGLEWIGRIDPENDETTYAPKFQGKATMTADTSSNTAYLQLTSLTSEDTAVYYCARSTVLDYWGHGTTLTVSSESARNPTIYPLTLPRALSSDPVIIGCLIHDYFPSGTMNVTWGKSGKDITTVNFPPALASGGGYTMSSQLTLPAVECPEGESVKCSVQHDSNAVQELDVKCSGPPPPCPPCPPSCHPSLSLQRPALEDLLLGSDASLTCTLNGLRNPEGAVFTWEPSTGKDAVQKKAVQNSCGCYSVSSVLPGCAERWNSGASFKCTVTHPESDTLTGTIAKITVNTFPPQVHLLPPPSEELALNELVSLTCLVRAFNPKEVLVRWLHGNEELSPESYLVFEPLKEPGEGATTYLVTSVLRVSAELWKQGDQYSCMVGHEALPMNFTQKTIDRLSGKPTNVSVSVIMSEGDGICY

SEQ ID NO: 40 - protein, 238 aa, Mus musculus
MKLPVRLLVLMFWIPGFSSDVLMTQTPLSLPVSLGDQASISCRASQSIVHTNGNTYLEWYLQKPGQSPKLLIYKVSNRFSGVPDRFSGSGSGTDFILKISRVEAEDLGVYYCFQGSHVPPTFGGGTKLEVKRADAAPTVSIFPPSSEQLTSGGASVVCFLNNFYPKDINVKWKIDGSERQNGVLNSWTDQDSKDSTYSMSSTLTLTKDEYERHNSYTCEATHKTSTSPIVKSFNRNEC

SEQ ID NO: 41 - protein, 5 aa, synthetic construct
NYYIH

SEQ ID NO: 42 - protein, 16 aa, synthetic construct
RIDPENNETTYAPKFQ

SEQ ID NO: 43 - protein, 16 aa, synthetic construct
RIDPENDQTTYAPKFQ

SEQ ID NO: 44 - protein, 16 aa, synthetic construct
RIDPENNQTTYAPKFQ

SEQ ID NO: 45 - protein, 134 aa, synthetic construct
MKCSWIIFFLMAVVTGVNSEVQLQQSGSELVKSGASVKLSCTVSGFNFTNYYIHWVRQRTEQGLEWIGRIDPENDETTYAPKFQGKATMTADTSSNTAYLQLTSLTSEDTAVYYCARSTVLDYWGHGTTLTVSS

SEQ ID NO: 46 - protein, 134 aa, synthetic construct
MKCSWIIFFLMAVVTGVNSEVQLQQSGSELVKSGASVKLSCTVSGFNFTDYYIHWVRQRTEQGLEWIGRIDPENNETTYAPKFQGKATMTADTSSNTAYLQLTSLTSEDTAVYYCARSTVLDYWGHGTTLTVSS

SEQ ID NO: 47 - protein, 134 aa, synthetic construct
MKCSWIIFFLMAVVTGVNSEVQLQQSGSELVKSGASVKLSCTVSGFNFTDYYIHWVRQRTEQGLEWIGRIDPENDQTTYAPKFQGKATMTADTSSNTAYLQLTSLTSEDTAVYYCARSTVLDYWGHGTTLTVSS

SEQ ID NO: 48 - protein, 134 aa, synthetic construct
MKCSWIIFFLMAVVTGVNSEVQLQQSGSELVKSGASVKLSCTVSGFNFTNYYIHWVRQRTEQGLEWIGRIDPENNETTYAPKFQGKATMTADTSSNTAYLQLTSLTSEDTAVYYCARSTVLDYWGHGTTLTVSS

SEQ ID NO: 49 - protein, 134 aa, synthetic construct
MKCSWIIFFLMAVVTGVNSEVQLQQSGSELVKSGASVKLSCTVSGFNFTNYYIHWVRQRTEQGLEWIGRIDPENDQTTYAPKFQGKATMTADTSSNTAYLQLTSLTSEDTAVYYCARSTVLDYWGHGTTLTVSS

SEQ ID NO: 50 - protein, 134 aa, synthetic construct
MKCSWIIFFLMAVVTGVNSEVQLQQSGSELVKSGASVKLSCTVSGFNFTDYYIHWVRQRTEQGLEWIGRIDPENNQTTYAPKFQGKATMTADTSSNTAYLQLTSLTSEDTAVYYCARSTVLDYWGHGTTLTVSS

SEQ ID NO: 51 - protein, 134 aa, synthetic construct
MKCSWIIFFLMAVVTGVNSEVQLQQSGSELVKSGASVKLSCTVSGFNFTNYYIHWVRQRTEQGLEWIGRIDPENNQTTYAPKFQGKATMTADTSSNTAYLQLTSLTSEDTAVYYCARSTVLDYWGHGTTLTVSS

SEQ ID NO: 52 - protein, 11 aa, synthetic construct
RSSQSIVHTNG

SEQ ID NO: 53 - protein, 13 aa, synthetic construct
SPASLSVSLGDRA

SEQ ID NO: 54 - protein, 13 aa, synthetic construct
SPASLSVSLGDRV

SEQ ID NO: 55 - protein, 13 aa, synthetic construct
SPASMSVSLGDRA

SEQ ID NO: 56 - protein, 13 aa, synthetic construct
TPLSLPVSLGDQA

SEQ ID NO: 57 - protein, 131 aa, synthetic construct
MKLPVRLLVLMFWIPGFSSDVLMTQSPASLSVSLGDRATISCRASQSIVHTNGNTYLEWYLQKPGQSPKLLIYKVSNRFSGVPDRFSGSGSGTDFILKISRVEAEDLGVYYCFQGSHVPPTFGGGTKLEVK

SEQ ID NO: 58 - protein, 131 aa, synthetic construct
MKLPVRLLVLMFWIPGFSSDVLMTQSPASLSVSLGDRVTISCRASQSIVHTNGNTYLEWYLQKPGQSPKLLIYKVSNRFSGVPDRFSGSGSGTDFILKISRVEAEDLGVYYCFQGSHVPPTFGGGTKLEVK

SEQ ID NO: 59 - protein, 131 aa, synthetic construct
MKLPVRLLVLMFWIPGFSSDVLMTQSPASLSVSLGDRVTISCRSSQSIVHTNGNTYLEWYLQKPGQSPKLLIYKVSNRFSGVPDRFSGSGSGTDFILKISRVEAEDLGVYYCFQGSHVPPTFGGGTKLEVK

SEQ ID NO: 60 - protein, 131 aa, synthetic construct
MKLPVRLLVLMFWIPGFSSDVLMTQSPASMSVSLGDRATISCRSSQSIVHTNGNTYLEWYLQKPGQSPKLLIYKVSNRFSGVPDRFSGSGSGTDFILKISRVEAEDLGVYYCFQGSHVPPTFGGGTKLEVK

SEQ ID NO: 61 - protein, 131 aa, synthetic construct
MKLPVRLLVLMFWIPGFSSDVLMTQSPASLSVSLGDRATISCRSSQSIVHTNGNTYLEWYLQKPGQSPKLLIYKVSNRFSGVPDRFSGSGSGTDFILKISRVEAEDLGVYYCFQGSHVPPTFGGGTKLEVK

SEQ ID NO: 62 - protein, 5 aa, synthetic construct
  VARIANT 1: note = X can be any neutral polar amino acid or acidic polar amino acid
XYYIH

SEQ ID NO: 63 - protein, 16 aa, synthetic construct
  VARIANT 7: note = X can be any neutral polar amino acid or acidic polar amino acid
  VARIANT 8: note = X can be any neutral polar amino acid or acidic polar amino acid
RIDPENXXTTYAPKFQ

SEQ ID NO: 64 - protein, 11 aa, synthetic construct
  VARIANT 2: note = X can be any nonpolar amino acid or neutral polar amino acid
RXSQSIVHTNG

SEQ ID NO: 65 - DNA, 1467 bp, Mus musculus
  source 1..1467: mol_type = other DNA
atggaatggatctggatctttctcttcatcctgtcaggaactgcaggtgtccaatcccaggttcagctgcagcagtctggagctgagctggcgaggcctggggcttcagtgaagctgtcctgcaaggcttctggctacaccttcacaagctatggtataagctgggtgaagcagagaactggacagggccttgagtggattggagagatttatcctagaagtggtaatacttactacaatgagaagttcaagggcaaggccacactgactgcagacaaatcctccagcacagcgtacatggagctccgcagcctgacatctgaggactctgcggtctatttctgtgcaagattggcatcgagctactacggtagtagctacgactggtacttcgatgtctggggcacagggaccacggtcaccgtctcctcagagtctgcgagaaatcccaccatctacccactgacactcccacgagctctgtcaagtgacccagtgataatcggctgcctgattcacgattacttcccttccggcacgatgaatgtgacctggggaaagagtgggaaggatataaccaccgtaaacttcccacctgccctggcctctgggggagggtacaccatgagcagccagttgaccctgccagctgtcgagtgcccagaaggagaatccgtgaaatgttccgtgcaacatgactctaacgccgtccaagaattggatgtgaagtgctctggtcctcctcctccttgtcctccttgtcctccttcctgccatcccagcctgtcactgcagcggccagctcttgaggacctgctcctgggttcagatgccagcctcacatgtactctgaatggcctgagaaatcctgagggagctgtcttcacctgggagccctccactgggaaggatgcagtgcagaagaaagctgtgcagaattcctgcggctgctacagtgtgtccagcgtcctgcctggctgtgctgagcgctggaacagtggcgcatcattcaagtgcacagttacccatcctgagtctgacaccttaactggcacaattgccaaaatcacagtgaacaccttcccaccccaggtccacctgctaccgccgccgtcggaggagctggccctgaatgagctcgtgtccctgacatgcctggtgcgagctttcaaccctaaagaagtgctggtgcgatggctgcatggaaatgaggagctgtccccagaaagctacctagtgtttgagcccctaaaggagccaggcgagggagccaccacctacctggtgacaagcgtgttgcgtgtatcagctgaactctggaaacagggtgaccagtactcctgcatggtgggccacgaggccttgcccatgaacttcacccagaagaccatcgaccgtctgtcgggtaaacccaccaatgtcagcgtgtctgtgatcatgtcagagggagatggcatctgctactga

SEQ ID NO: 66 - DNA, 705 bp, Mus musculus
  source 1..705: mol_type = other DNA
atgaggacccctgctcagtttcttggaatcttgttgctctggtttccaggtatcaaatgtgacatcaagatgacccagtctccatcttccatgtatgcatctctaggagagagagtcactatcacttgcaaggcgagtcaggacattaatagctatttaagctggttccagcagaaaccagggaaatctcctaagaccctgatctatcgtgcaaacagattggtagatggggtcccatcaaggttcagtggcagtggatctgggcaagattattctctcaccatcagcagcctggagtatgaagatatgggaatttattattgtctacagtatgatgagtttccgctcacgttcggtgctgggaccaagctggagctgaaacgggctgatgctgcaccaactgtatccatcttcccaccatccagtgagcagttaacatctggaggtgcctcagtcgtgtgcttcttgaacaacttctaccccaaagacatcaatgtcaagtggaagattgatggcagtgaacgacaaaatggcgtcctgaacagttggactgatcaggacagcaaagacagcacctacagcatgagcagcaccctcacgttgaccaaggacgagtatgaacgacataacagctatacctgtgaggccactcacaagacatcaacttcacccattgtcaagagcttcaacaggaatgagtgttga

SEQ ID NO: 67 - DNA, 1440 bp, Mus musculus
  source 1..1440: mol_type = other DNA
atgggcaggcttacttcttcattcctgttactgattgtccctgcatatgtcctgtcccaggttactctgaaagagtctggccctgggatattgcagccctcccagaccctcagtctgacttgttctttctctgggttttcactgagcacttttggtatgggtgtaggctggattcgtcagccttcagggaagggtctggagtggctggcacacatttggtgggatgatgataagtactataacccagccctgaagagtcggctcacaatctccaaggatacctccaaaaaccaggtattcctcaagatcgccaatgtggacactgcagatactgccacatactactgtgctcgaatagctgggtttgactactggggccaaggcaccactctcacagtctcctcagagtctgcgagaaatcccaccatctacccactgacactcccacgagctctgtcaagtgacccagtgataatcggctgcctgattcacgattacttcccttccggcacgatgaatgtgacctggggaaagagtgggaaggatataaccaccgtaaacttcccacctgccctggcctctgggggagggtacaccatgagcagccagttgaccctgccagctgtcgagtgcccagaaggagaatccgtgaaatgttccgtgcaacatgactctaacgccgtccaagaattggatgtgaagtgctctggtcctcctcctccttgtcctccttgtcctccttcctgccatcccagcctgtcactgcagcggccagctcttgaggacctgctcctgggttcagatgccagcctcacatgtactctgaatggcctgagaaatcctgagggagctgtcttcacctgggagccctccactgggaaggatgcagtgcagaagaaagctgtgcagaattcctgcggctgctacagtgtgtccagcgtcctgcctggctgtgctgagcgctggaacagtggcgcatcattcaagtgcacagttacccatcctgagtctgacaccttaactggcacaattgccaaaatcacagtgaacaccttcccaccccaggtccacctgctaccgccgccgtcggaggagctggccctgaatgagctcgtgtccctgacatgcctggtgcgagctttcaaccctaaagaagtgctggtgcgatggctgcatggaaatgaggagctgtccccagaaagctacctagtgtttgagcccctaaaggagccaggcgagggagccaccacctacctggtgacaagcgtgttgcgtgtatcagctgaactctggaaacagggtgaccagtactcctgcatggtgggccacgaggccttgcccatgaacttcacccagaagaccatcgaccgtctgtcgggtaaacccaccaatgtcagcgtgtctgtgatcatgtcagagggagatggcatctgctactga

SEQ ID NO: 68 - DNA, 708 bp, Mus musculus
  source 1..708: mol_type = other DNA
atgcattttcaagtgcagattttcagcttcctgctaatcagtgcctcagtcataatgtccagaggacaaattgttctcacccagtctccagcaatcatgtctgcatctccaggggagaaggtcaccataacctgcagtgccagctcaagtgtaagttacatgcactggttccagcagaagccaggcacttctcccaaactctggatttatagcacatccaacctggcttctggagtccctgctcgcttcagtggcagtggatctgggacctcttactctctcacaatcagccgaatggaggctgaagatgctgccacttattactgccagcaaaggagtagttacccgtacacgttcggaggggggaccaagctggaaataaaacgggctgatgctgcaccaactgtatccatcttcccaccatccagtgagcagttaacatctggaggtgcctcagtcgtgtgcttcttgaacaacttctaccccaaagacatcaatgtcaagtggaagattgatggcagtgaacgacaaaatggcgtcctgaacagttggactgatcaggacagcaaagacagcacctacagcatgagcagcaccctcacgttgaccaaggacgagtatgaacgacataacagctatacctgtgaggccactcacaagacatcaacttcacccattgtcaagagcttcaacaggaatgagtgttga

SEQ ID NO: 69 - DNA, 1446 bp, Mus musculus
  source 1..1446: mol_type = other DNA
atgggattcagcaggatctttctcttcctcctgtcagtaactacaggtgtccactcccaggcttatctacagcagtctggggctgagctggtgaggcctggggcctcagtgaggatgtcctgcaaggcttctgactacacatttaccagttacaatatccactgggtaaagcagacacctagacagggcctggaatggattggagctatttattcaggaaatggtgctacttcccacaatcagaagttcaagggcagggccacactgactgtagacaaatcctccagcacagcctacatgcaactcagcagcctgacatctgaagactctgcggtctatttctgtacaagagtgggactccggtccccttttgacttctggggccaaggcaccactctcacagtctcctcagagtctgcgagaaatcccaccatctacccactgacactcccacgagctctgtcaagtgacccagtgataatcggctgcctgattcacgattacttcccttccggcacgatgaatgtgacctggggaaagagtgggaaggatataaccaccgtaaacttcccacctgccctggcctctgggggagggtacaccatgagcagccagttgaccctgccagctgtcgagtgcccagaaggagaatccgtgaaatgttccgtgcaacatgactctaacgccgtccaagaattggatgtgaagtgctctggtcctcctcctccttgtcctccttgtcctccttcctgccatcccagcctgtcactgcagcggccagctcttgaggacctgctcctgggttcagatgccagcctcacatgtactctgaatggcctgagaaatcctgagggagctgtcttcacctgggagccctccactgggaaggatgcagtgcagaagaaagctgtgcagaattcctgcggctgctacagtgtgtccagcgtcctgcctggctgtgctgagcgctggaacagtggcgcatcattcaagtgcacagttacccatcctgagtctgacaccttaactggcacaattgccaaaatcacagtgaacaccttcccaccccaggtccacctgctaccgccgccgtcggaggagctggccctgaatgagctcgtgtccctgacatgcctggtgcgagctttcaaccctaaagaagtgctggtgcgatggctgcatggaaatgaggagctgtccccagaaagctacctagtgtttgagcccctaaaggagccaggcgagggagccaccacctacctggtgacaagcgtgttgcgtgtatcagctgaactctggaaacagggtgaccagtactcctgcatggtgggccacgaggccttgcccatgaacttcacccagaagaccatcgaccgtctgtcgggtaaacccaccaatgtcagcgtgtctgtgatcatgtcagagggagatggcatctgctactga

SEQ ID NO: 70 - DNA, 705 bp, Mus musculus
  source 1..705: mol_type = other DNA
atggagtcacagactcaggtctttgtatacatgttgctgtggttgtctggtgttgatggagacattgtgatgacccagtctctaaaattcatgtccacatcgggaggagacagggtcagcgtcacctgcaaggccagtcagagtgtgggtacaagtgtagcctggtatcagcagaaaccaggacaatctcctaaaccactgatttattcggcatcttatcggtacagtggagtccctgatcgcttcacaggcagtggatctgggacagatttcagtctcaccatcagcaatgtgcagtctgaagacttggcagaatatttctgtcagcaatataacaactatccgtacacgttcggaggggggaccaagctggagataaaacgggctgatgctgcaccaactgtatccatcttcccaccatccagtgagcagttaacatctggaggtgcctcagtcgtgtgcttcttgaacaacttctaccccaaagacatcaatgtcaagtggaagattgatggcagtgaacgacaaaatggcgtcctgaacagttggactgatcaggacagcaaagacagcacctacagcatgagcagcaccctcacgttgaccaaggacgagtatgaacgacataacagctatacctgtgaggccactcacaagacatcaacttcacccattgtcaagagcttcaacaggaatgagtgttga

SEQ ID NO: 71 - DNA, 1437 bp, Mus musculus
  source 1..1437: mol_type = other DNA
atgaaatgcagctggatcatcttcttcctgatggcagtggttacaggggtcaattcagaggttcagctgcagcagtctgggtcagagcttgtgaagtctggggcctcagtcaagttgtcctgcacagtttctgggttcaactttacagactactatatacactgggtgaggcagaggactgaacagggcctggaatggattggaaggattgatcctgagaatgatgaaactacatatgccccgaaattccagggcaaggccactatgacagcagacacatcttccaacacagcctacctgcagctcaccagcctgacatctgaagacactgccgtctattactgtgctagatctacggtccttgactactggggccacggcaccactctcacagtctcctcagagtctgcgagaaatcccaccatctacccactgacactcccacgagctctgtcaagtgacccagtgataatcggctgcctgattcacgattacttcccttccggcacgatgaatgtgacctggggaaagagtgggaaggatataaccaccgtaaacttcccacctgccctggcctctgggggagggtacaccatgagcagccagttgaccctgccagctgtcgagtgcccagaaggagaatccgtgaaatgttccgtgcaacatgactctaacgccgtccaagaattggatgtgaagtgctctggtcctcctcctccttgtcctccttgtcctccttcctgccatcccagcctgtcactgcagcggccagctcttgaggacctgctcctgggttcagatgccagcctcacatgtactctgaatggcctgagaaatcctgagggagctgtcttcacctgggagccctccactgggaaggatgcagtgcagaagaaagctgtgcagaattcctgcggctgctacagtgtgtccagcgtcctgcctggctgtgctgagcgctggaacagtggcgcatcattcaagtgcacagttacccatcctgagtctgacaccttaactggcacaattgccaaaatcacagtgaacaccttcccaccccaggtccacctgctaccgccgccgtcggaggagctggccctgaatgagctcgtgtccctgacatgcctggtgcgagctttcaaccctaaagaagtgctggtgcgatggctgcatggaaatgaggagctgtccccagaaagctacctagtgtttgagcccctaaaggagccaggcgagggagccaccacctacctggtgacaagcgtgttgcgtgtatcagctgaactctggaaacagggtgaccagtactcctgcatggtgggccacgaggccttgcccatgaacttcacccagaagaccatcgaccgtctgtcgggtaaacccaccaatgtcagcgtgtctgtgatcatgtcagagggagatggcatctgctactga

SEQ ID NO: 72 - DNA, 717 bp, Mus musculus
  source 1..717: mol_type = other DNA
atgaagttgcctgttaggctgttggtgctgatgttctggattcctggattcagcagtgatgttttgatgacccaaactccactctccctgcctgtcagtcttggagatcaagcctccatctcttgtagagctagtcagagcattgtacacactaatgggaacacctatttagaatggtacctgcagaaaccaggccagtctccaaagctcctgatctacaaagtttccaaccgattttctggggtcccagacaggttcagtggcagtggatctgggacagatttcatactcaagatcagcagagtggaggctgaggatctgggagtttattactgctttcaaggttcacatgttcctccgacgttcggtggaggcaccaagctggaagtcaaacgggctgatgctgcaccaactgtatccatcttcccaccatccagtgagcagttaacatctggaggtgcctcagtcgtgtgcttcttgaacaacttctaccccaaagacatcaatgtcaagtggaagattgatggcagtgaacgacaaaatggcgtcctgaacagttggactgatcaggacagcaaagacagcacctacagcatgagcagcaccctcacgttgaccaaggacgagtatgaacgacataacagctatacctgtgaggccactcacaagacatcaacttcacccattgtcaagagcttcaacaggaatgagtgttag

SEQ ID NO: 73 - DNA, 1374 bp, Mus musculus
  source 1..1374: mol_type = other DNA
atgaaatgcagctggatcatcttcttcctgatggcagtggttacaggggtcaattcagaggttcagctgcagcagtctgggtcagagcttgtgaagtctggggcctcagtcaagttgtcctgcacagtttctgggttcaactttacagactactatatacactgggtgaggcagaggactgaacagggcctggaatggattggaaggattgatcctgagaatgatgaaactacatatgccccgaaattccagggcaaggccactatgacagcagacacatcttccaacacagcctacctgcagctcaccagcctgacatctgaagacactgccgtctattactgtgctagatctacggtccttgactactggggccacggcaccactctcacagtctcctcaaaaacgacacccccatctgtctatccactggcccctggatctgctgcccaaactaactccatggtgaccctgggatgcctggtcaagggctatttccctgagccagtgacagtgacctggaactctggatccctgtccagcggtgtgcacaccttcccagctgtcctgcagtctgacctctacactctgagcagctcagtgactgtcccctccagcacctggcccagcgagaccgtcacctgcaacgttgcccacccggccagcagcaccaaggtggacaagaaaattgtgcccagggattgtggttgtaagccttgcatatgtacagtcccagaagtatcatctgtcttcatcttccccccaaagcccaaggatgtgctcaccattactctgactcctaaggtcacgtgtgttgtggtagacatcagcaaggatgatcccgaggtccagttcagctggtttgtagatgatgtggaggtgcacacagctcagacgcaaccccgggaggagcagttcaacagcactttccgctcagtcagtgaacttcccatcatgcaccaggactggctcaatggcaaggagttcaaatgcagggtcaacagtgcagctttccctgcccccatcgagaaaaccatctccaaaaccaaaggcagaccgaaggctccacaggtgtacaccattccacctcccaaggagcagatggccaaggataaagtcagtctgacctgcatgataacagacttcttccctgaagacattactgtggagtggcagtggaatgggcagccagcggagaactacaagaacactcagcccatcatggacacagatggctcttacttcgtctacagcaagctcaatgtgcagaagagcaactgggaggcaggaaatactttcacctgctctgtgttacatgagggcctgcacaaccaccatactgagaagagcctctcccactctcctggtaaataa

SEQ ID NO: 74 - DNA, 1407 bp, synthetic construct
  source 1..1407: mol_type = other DNA
atgaaatgcagctggatcatcttcttcctgatggcagtggttacaggggtcaattcagaggttcagctgcagcagtctgggtcagagcttgtgaagtctggggcctcagtcaagttgtcctgcacagtttctgggttcaactttacagactactatatacactgggtgaggcagaggactgaacagggcctggaatggattggaaggattgatcctgagaatgatgaaactacatatgccccgaaattccagggcaaggccactatgacagcagacacatcttccaacacagcctacctgcagctcaccagcctgacatctgaagacactgccgtctattactgtgctagatctacggtccttgactactggggccacggcaccactctcacagtctcctcagcatccccgactagttccaccaagggcccatcggtcttccccctggcaccctcctccaagagcacctctgggggcacagcggccctgggctgcctggtcaaggactacttccccgaaccggtgacggtgtcgtggaactcaggcgccctgaccagcggcgtgcacaccttcccggctgtcctacagtcctcaggactctactccctcagcagcgtggtgaccgtgccctccagcagcttgggcacccagacctacatctgcaacgtgaatcacaagcccagcaacaccaaggtggacaagaaagttgagcccaaatcttgtgacaaaactcacacatgcccaccgtgcccagcacctgaactcctggggggaccgtcagtcttcctcttccccccaaaacccaaggacaccctcatgatctcccggacccctgaggtcacatgcgtggtggtggacgtgagccacgaagaccctgaggtcaagttcaactggtacgtggacggcgtggaggtgcataatgccaagacaaagccgcgggaggagcagtacaacagcacgtaccgtgtggtcagcgtcctcaccgtcctgcaccaggactggctgaatggcaaggagtacaagtgcaaggtctccaacaaagccctcccagcccctatcgagaaaaccatctccaaagccaaagggcagccccgagaaccacaggtgtacaccctgcccccatcccgggatgagctgaccaagaaccaggtcagcctgacctgcctggtcaaaggcttctatcccagcgacatcgccgtggagtgggagagcaatgggcagccggagaacaactacaagaccacgcctcccgtgctggactccgacggctccttcttcctctacagcaagctcaccgtggacaagagcaggtggcagcaggggaacgtcttctcatgctccgtgatgcatgagggtctgcacaaccactacacgcagaagagcctctccctgtctccgggtaaatga

SEQ ID NO: 75 - DNA, 723 bp, synthetic construct
  source 1..723: mol_type = other DNA
atggacatgaagttgcctgttaggctgttggtgctgatgttctggattcctggattcagcagtgatgttttgatgacccaaactccactctccctgcctgtcagtcttggagatcaagcctccatctcttgtagagctagtcagagcattgtacacactaatgggaacacctatttagaatggtacctgcagaaaccaggccagtctccaaagctcctgatctacaaagtttccaaccgattttctggggtcccagacaggttcagtggcagtggatctgggacagatttcatactcaagatcagcagagtggaggctgaggatctgggagtttattactgctttcaaggttcacatgttcctccgacgttcggtggaggcaccaagctggaagtcaaacgggctgatgctgcaccaactgtatccatcttcccaccatccagtgagcagttaacatctggaggtgcctctgttgtgtgcctgctgaataacttctatcctcgagaggccaaagtacagtggaaggtggataacgccctccaatcgggtaactcccaggagagtgtcacagagcaggacagcaaggacagcacctacagcctcagcagcaccctgacgctgagcaaagcagactacgagaaacacaaagtctacgcctgcgaagtcacccatcagggcctgagctcgcccgtcacaaagagcttcaacaggggagagtgttag

SEQ ID NO: 76 - protein, 457 aa, Mus musculus
MKCSWIIFFLMAVVTGVNSEVQLQQSGSELVKSGASVKLSCTVSGFNFTDYYIHWVRQRTEQGLEWIGRIDPENDETTYAPKFQGKATMTADTSSNTAYLQLTSLTSEDTAVYYCARSTVLDYWGHGTTLTVSSKTTPPSVYPLAPGSAAQTNSMVTLGCLVKGYFPEPVTVTWNSGSLSSGVHTFPAVLQSDLYTLSSSVTVPSSTWPSETVTCNVAHPASSTKVDKKIVPRDCGCKPCICTVPEVSSVFIFPPKPKDVLTITLTPKVTCVVVDISKDDPEVQFSWFVDDVEVHTAQTQPREEQFNSTFRSVSELPIMHQDWLNGKEFKCRVNSAAFPAPIEKTISKTKGRPKAPQVYTIPPPKEQMAKDKVSLTCMITDFFPEDITVEWQWNGQPAENYKNTQPIMDTDGSYFVYSKLNVQKSNWEAGNTFTCSVLHEGLHNHHTEKSLSHSPGK

SEQ ID NO: 77 - protein, 468 aa, synthetic construct
MKCSWIIFFLMAVVTGVNSEVQLQQSGSELVKSGASVKLSCTVSGFNFTDYYIHWVRQRTEQGLEWIGRIDPENDETTYAPKFQGKATMTADTSSNTAYLQLTSLTSEDTAVYYCARSTVLDYWGHGTTLTVSSASPTSSTKGPSVFPLAPSSKSTSGGTAALGCLVKDYFPEPVTVSWNSGALTSGVHTFPAVLQSSGLYSLSSVVTVPSSSLGTQTYICNVNHKPSNTKVDKKVEPKSCDKTHTCPPCPAPELLGGPSVFLFPPKPKDTLMISRTPEVTCVVVDVSHEDPEVKFNWYVDGVEVHNAKTKPREEQYNSTYRVVSVLTVLHQDWLNGKEYKCKVSNKALPAPIEKTISKAKGQPREPQVYTLPPSRDELTKNQVSLTCLVKGFYPSDIAVEWESNGQPENNYKTTPPVLDSDGSFFLYSKLTVDKSRWQQGNVFSCSVMHEGLHNHYTQKSLSLSPGK

SEQ ID NO: 78 - protein, 240 aa, synthetic construct
MDMKLPVRLLVLMFWIPGFSSDVLMTQTPLSLPVSLGDQASISCRASQSIVHTNGNTYLEWYLQKPGQSPKLLIYKVSNRFSGVPDRFSGSGSGTDFILKISRVEAEDLGVYYCFQGSHVPPTFGGGTKLEVKRADAAPTVSIFPPSSEQLTSGGASVVCLLNNFYPREAKVQWKVDNALQSGNSQESVTEQDSKDSTYSLSSTLTLSKADYEKHKVYACEVTHQGLSSPVTKSFNRGEC

SEQ ID NO: 79 - protein, 5 aa, synthetic construct
  VARIANT 1: note = X can be Asparagine or Aspartic Acid
XYYIH

SEQ ID NO: 80 - protein, 16 aa, synthetic construct
  VARIANT 7: note = X can be Asparagine or Aspartic Acid
  VARIANT 8: note = X can be Glutamine or Glutamic Acid
RIDPENXXTTYAPKFQ

SEQ ID NO: 81 - protein, 11 aa, synthetic construct
  VARIANT 2: note = X can be Alanine or Serine
RXSQSIVHTNG

SEQ ID NO: 82 - protein, 13 aa, synthetic construct
  VARIANT 5: note = X can be non-polar amino acid
  VARIANT 13: note = X can be non-polar amino acid
SPASXSVSLGDRX

SEQ ID NO: 83 - protein, 13 aa, synthetic construct
  VARIANT 5: note = X can be Leucine or Methionine
  VARIANT 13: note = X can be Alanine or Valine
SPASXSVSLGDRX

SEQ ID NO: 84 - DNA, 36 bp, synthetic construct
  source 1..36: mol_type = other DNA
gtggtggaattcaccatgatgaaaaaaccagttgct

SEQ ID NO: 85 - DNA, 36 bp, synthetic construct
  source 1..36: mol_type = other DNA
gaagggccctctagattttgaaataagtgaatgacc

SEQ ID NO: 86 - DNA, 36 bp, synthetic construct
  source 1..36: mol_type = other DNA
gatgttggtctacctgatggtcaaatgggaaattca

SEQ ID NO: 87 - DNA, 36 bp, synthetic construct
  source 1..36: mol_type = other DNA
aagaccactagcatttatcaatgtgtttggatactc

SEQ ID NO: 88 - DNA, 36 bp, synthetic construct
  source 1..36: mol_type = other DNA
aaaactcaacttagagctgctgaaactgaaaagtat

SEQ ID NO: 89 - DNA, 36 bp, synthetic construct
  source 1..36: mol_type = other DNA
tccatttttagctagatactcacctagagtgttggc

SEQ ID NO: 90 - DNA, 36 bp, synthetic construct
  source 1..36: mol_type = other DNA
gtattaaactttgcaaatcctgatatggtaggtcat

SEQ ID NO: 91 - DNA, 36 bp, synthetic construct
  source 1..36: mol_type = other DNA
tataaagtcaaacttatcttctcctagtttatctaa

SEQ ID NO: 92 - DNA, 36 bp, synthetic construct
  source 1..36: mol_type = other DNA
atggaagcggcggttaaggctgttgaaactgtagat

SEQ ID NO: 93 - DNA, 36 bp, synthetic construct
  source 1..36: mol_type = other DNA
gctgaccacggtaacgctgaatatatgttagaccca

SEQ ID NO: 94 - DNA, 36 bp, synthetic construct
  source 1..36: mol_type = other DNA
accaacctgccagttccatttattgtagttggtcaa

SEQ ID NO: 95 - DNA, 36 bp, synthetic construct
  source 1..36: mol_type = other DNA
aaactttctgacatcgcaccgactgttttagatatg

SEQ ID NO: 96 - DNA, 36 bp, synthetic construct
  source 1..36: mol_type = other DNA
gtggtggaattcaccatgttggtttctaaaaaacct

SEQ ID NO: 97 - DNA, 36 bp, synthetic construct
  source 1..36: mol_type = other DNA
gaagggccctctagattccacgatgaacagcggctt

SEQ ID NO: 98 - DNA, 36 bp, synthetic construct
  source 1..36: mol_type = other DNA
aatgctagtggtcttgaagtcggtctgcctgaccgt

SEQ ID NO: 99 - DNA, 36 bp, synthetic construct
  source 1..36: mol_type = other DNA
cagaccggaagcgtcgatcagaggtagaccaacatc

SEQ ID NO: 100 - DNA, 36 bp, synthetic construct
  source 1..36: mol_type = other DNA
ctagctaaaaatggaaaaactcagttgcgtatttcc

SEQ ID NO: 101 - DNA, 36 bp, synthetic construct
  source 1..36: mol_type = other DNA
gtcgtttttcgccatccactctctaagttgagtttt

SEQ ID NO: 102 - DNA, 36 bp, synthetic construct
  source 1..36: mol_type = other DNA
aagtttgactttataatctgtaactatccgaacggc

SEQ ID NO: 103 - DNA, 36 bp, synthetic construct
  source 1..36: mol_type = other DNA
aatggtgtcgtatttgccgcttgcaaagtttaatac

SEQ ID NO: 104 - DNA, 17 bp, synthetic construct
  source 1..17: mol_type = other DNA
sargtnmagctgsagtc

SEQ ID NO: 105 - DNA, 23 bp, synthetic construct
  source 1..23: mol_type = other DNA
sargtnmagctgsagsagtcwgg

SEQ ID NO: 106 - DNA, 21 bp, synthetic construct
  source 1..21: mol_type = other DNA
caggttactctgaaagwtstg

SEQ ID NO: 107 - DNA, 20 bp, synthetic construct
  source 1..20: mol_type = other DNA
gaggtccarctgcaacartc

SEQ ID NO: 108 - DNA, 20 bp, synthetic construct
  source 1..20: mol_type = other DNA
caggtccaactvcagcarcc

SEQ ID NO: 109 - DNA, 20 bp, synthetic construct
  source 1..20: mol_type = other DNA
gaggtgaasstggtggaatc

SEQ ID NO: 110 - DNA, 20 bp, synthetic construct
  source 1..20: mol_type = other DNA
gatgtgaacttggaagtgtc

SEQ ID NO: 111 - DNA, 22 bp, synthetic construct
  source 1..22: mol_type = other DNA
gatggtgggatttctcgcagac

SEQ ID NO: 112 - DNA, 32 bp, synthetic construct
  source 1..32: mol_type = other DNA
ggctgcagsttcagtggcagtggrtcwggrac

SEQ ID NO: 113 - DNA, 21 bp, synthetic construct
  source 1..21: mol_type = other DNA
aacgtgagggtgctgctcatg